European Patent Application EP 4 116 416 A1, published January 11, 2023. Title: A novel serine protease variant. Applicant: CJ CheilJedang Corporation. The sequence listing filed with the application follows.

SEQUENCE LISTING (72 sequences)

SEQ ID NO: 1 - DNA, 6922 bp, Artificial Sequence
  pBE-S-TFP
actagtgttcttttctgtatgaaaatagttatttcgagtctctacggaaatagcgagagatgatatacctaaatagagataaaatcatctcaaaaaaatgggtctactaaaatattattccatctattacaataaattcacagaatagtcttttaagtaagtctactctgaacttaagcaaaaggagagggacgcgtgtgagaagcaaaaaattgtggatcagcttgttgtttgcgttaacgttaatctttacgatggcgttcagcaacatgtctgcgcaggctgcggccggtgcacatatgcaagagctggcgttgaaacgggacctcggcctctctgacgcagaagtagccgaactccgggctgctgaggcggaagcggtcgagctcgaggaggagctccgcgattcattagggtcagacttcggcggtgtatatctggatgctgacaccaccgaaattacggtcgcggtaaccgacccggcagcggtaagtcgtgtcgacgcggatgatgtcacagttgatgttgtcgatttcggggaaacagctttgaatgattttgtggcttcattaaatgccattgccgacacggcagaccctaaagtcactggatggtataccgatctcgaaagtgatgccgtagtcattacgaccttgcgtggcgggactcctgctgccgaggaacttgctgagagagcgggtctcgacgaaagagccgttcggattgtggaagaagatgaagaaccacagagcttggctgcaattattggtggaaacccgtactatttcggaaattacagatgcagtatcgggtttagtgtccgtcagggctctcaaacgggattcgcgaccgcaggccactgcggatccacggggacgcgtgtgtcttctccttcaggaacagttgcaggaagttatttcccgggtcgcgatatgggctgggtgcggattacatcagcagatactgtaacaccactcgtaaatcggtataatgggggaactgttacggtcactgggtcacaagaagctgccaccggatcctccgtttgtcgctctggagcaacaacgggctggcgctgcggaactatccaatcaaaaaaccaaacggttcgctatgcagaagggactgttactggtttaacaagaactacagcctgtgctgaaggtggggattctggagggccatggctcacaggtagccaggcgcaaggggttacaagcggcggaacaggcgattgcagaagtggagggattacctttttccaaccaatcaatccattgcttagctatttcggccttcaattagtgaccggctgaaagcttgtcgacctgcagtctagacatcaccatcatcaccactaatgcggtagtttatcacagttaaattgctaacgcagtcaggcaccgtgtatgaaatctaacaatgcgctcatcgtcatcctcggcaccgtcaccctggatgctgtaggcataggcttggttatgccggtactgccgggcctatttcactttttgcattctacaaactgcataactattatgtaaatcgctcctttttaggtggcacaaatgtgaggcattttcgctctttccggcaaccacttccaagtaaagtataacacactatactttatattcataaagtgtgtgctctgcgaggctgtcggcagtgccgaccaaaaccataaaacctttaagacctttcttttttttacgagaaaaaagaaacaaaaaaacctgccctctgccacctcagcaaaggggggttttgctctcgtgctcgtttaaaaatcagcaagggacaggtagtattttttgagaagatcactcaaaaaatctccacctttaaacccttgccaatttttattttgtccgttttgtctagcttaccgaaagccagactcagcaagaataaaatttttattgtctttcggttttctagtgtaacggacaaaaccactcaaaataaaaaagatacaagagaggtctctcgtatcttttattcagcaatcgcgcccgattgctgaacagattaataatagattttagctttttatttgttgaaaaaagctaatcaaattgttgtcgggatcaattactgcaaagtctcgttcatcccaccactgatcttttaatgatgtattggggtgcaaaatgcccaaaggcttaatatgttgatataattcatcaattccctctacttcaatgcggcaactagcagtaccagcaataaacgactccgcacctgtacaaaccggtgaatcattactacgagagcgccagccttcatcacttgcctcccatagatgaatccgaacctcattacacattagaactgcgaatccatcttcatggtgaaccaaagtgaaacctagtttatcgcaataaaaacctatactctttttaatatccccgactggcaatgccgggatagactgtaacattctcacgcataaaatcccctttcattttctaatgtaaatctattaccttattattaattcaattcgctcataattaatcctttttcttattacgcaaaatggcccgatttaagcacaccctttattccgttaatgcgccatgacagccatgataattactaatactaggagaagttaataaatacgagcaaaaggccagcaaaaggccaggaaccgtaaaaaggccgcgttgctggcgtttttccataggctccgcccccctgacgagcatcacaaaaatcgacgctcaagtcagaggtggcgaaacccgacaggactataaagataccaggcgtttccccctggaagctccctcgtgcgctctcctgttccgaccctgccgcttaccggatacctgtccgcctttctcccttcgggaagcgtggcgctttctcatagctcacgctgtaggtatctcagttcggtgtaggtcgttcgctccaagctgggctgtgtgcacgaaccccccgttcagcccgaccgctgcgccttatccggtaactatcgtcttgagtccaacccggtaagacacgacttatcgccactggcagcagccactggtaacaggattagcagagcgaggtatgtaggcggtgctacagagttcttgaagtggtggcctaactacggctacactagaagaacagtatttggtatctgcgctctgctgaagccagttaccttcggaaaaagagttggtagctcttgatccggcaaacaaaccaccgctggtagcggtggtttttttgtttgcaagcagcagattacgcgcagaaaaaaaggatctcaagaagatcctttgatcttttctacggggtctgacgctcagtggaacgaaaactcacgttaagggattttggtcatgagattatcaaaaaggatcttcacctagatccttttaaattaaaaatgaagttttaaatcaatctaaagtatatatgagtaaacttggtctgacagttaccaatgcttaatcagtgaggcacctatctcagcgatctgtctatttcgttcatccatagttgcctgactccccgtcgtgtagataactacgatacgggagggcttaccatctggccccagtgctgcaatgataccgcgagacccacgctcaccggctccagatttatcagcaataaaccagccagccggaagggccgagcgcagaagtggtcctgcaactttatccgcctccatccagtctattaattgttgccgggaagctagagtaagtagttcgccagttaatagtttgcgcaacgttgttgccattgctacaggcatcgtggtgtcacgctcgtcgtttggtatggcttcattcagctccggttcccaacgatcaaggcgagttacatgatcccccatgttgtgcaaaaaagcggttagctccttcggtcctccgatcgttgtcagaagtaagttggccgcagtgttatcactcatggttatggcagcactgcataattctcttactgtcatgccatccgtaagatgcttttctgtgactggtgagtactcaaccaagtcattctgagaatagtgtatgcggcgaccgagttgctcttgcccggcgtcaatacgggataataccgcgccacatagcagaactttaaaagtgctcatcattggaaaacgttcttcggggcgaaaactctcaaggatcttaccgctgttgagatccagttcgatgtaacccactcgtgcacccaactgatcttcagcatcttttactttcaccagcgtttctgggtgagcaaaaacaggaaggcaaaatgccgcaaaaaagggaataagggcgacacggaaatgttgaatactcatactcttcctttttcaatattattgaagcatttatcagggttattgtctcatgagcggatacatatttgaatgtatttagaaaaataaacaaataggggttccgcgcacatttccccgaaaagtgccacctgacgtctaagaaaccattattatcatgacattaacctataaaaataggcgtatcacgaggccctttcgtctcgcgcgtttcggtgatgacggtgaaaacctctgacagtaaccaacatgattaacaattattagaggtcatcgttcaaaatggtatgcgttttgacacatccactatatatccgtgtcgttctgtccactcctgaatcccattccagaaattctctagcgattccagaagtttctcagagtcggaaagttgaccagacattacgaactggcacagatggtcataacctgaaggaagatctgattgcttaactgcttcagttaagaccgaagcgctcgtcgtataacagatgcgatgatgcagaccaatcaacatggcacctgccattgctacctgtacagtcaaggatggtagaaatgttgtcggtccttgcacacgaatattacgccatttgcctgcatattcaaacagctcttctacgataagggcacaaatcgcatcgtggaacgtttgggcttctaccgatttagcagtttgatacactttctctaagtatccacctgaatcataaatcggcaaaatagagaaaaattgaccatgtgtaagcggccaatctgattccacctgagatgcataatctagtagaatctcttcgctatcaaaattcacttccaccttccactcaccggttgtccattcatggctgaactctgcttcctctgttgacatgacacacatcatctcaatatccgaatagggcccatcagtctgacgaccaagagagccataaacaccaatagccttaacatcatccccatatttatccaatattcgttccttaatttcatgaacaatcttcattctttcttctctagtcattattattggtccattcactattctcattcccttttcagataattttagatttgcttttctaaataagaatatttggagagcaccgttcttattcagctattaataactcgtcttcctaagcatccttcaatccttttaataacaattatagcatctaatcttcaacaaactggcccgtttgttgaactactctttaataaaataatttttccgttcccaattccacattgcaataatagaaaatccatcttcatcggctttttcgtcatcatctgtatgaatcaaatcgccttcttctgtgtcatcaaggtttaattttttatgtatttcttttaacaaaccaccataggagattaaccttttacggtgtaaaccttcctccaaatcagacaaacgtttcaaattcttttcttcatcatcggtcataaaatccgtatcctttacaggatattttgcagtttcgtcaattgccgattgtatatccgatttatatttatttttcggtcgaatcatttgaacttttacatttggatcatagtctaatttcattgcctttttccaaaattgaatccattgtttttgattcacgtagttttctgtattcttaaaataagttggttccacacataccaatacatgcatgtgctgattataagaattatctttattatttattgtcacttccgttgcacgcataaaaccaacaagatttttattaatttttttatattgcatcattcggcgaaatccttgagccatatctgacaaactcttatttaattcttcgccatcataaacatttttaactgttaatgtgagaaacaaccaacgaactgttggcttttgtttaataacttcagcaacaaccttttgtgactgaatgccatgtttcattgctctcctccagttgcacattggacaaagcctggatttacaaaaccacactcgatacaactttctttcgcctgtttcacgattttgtttatactctaatatttcagcacaatcttttactctttcagcctttttaaattcaagaatatgcagaagttcaaagtaatcaacattagcgattttcttttctctccatggtctcacttttccactttttgtcttgtccactaaaacccttgatttttcatctgaataaatgctactattaggacacataatattaaaagaaacccccatctatttagttatttgtttagtcacttataactttaacagatggggtttttctgtgcaaccaattttaagggttttcaatactttaaaacacatacataccaacacttcaacgcacctttcagcaactaaaataaaaatgacgttatttctatatgtatcaagataagaaagaacaagttcaaaaccatcaaaaaaagacaccttttcaggtgctttttttattttataaactcattccctgatctcgacttcgttctttttttacctctcggttatgagttagttcaaattcgttctttttaggttctaaatcgtgtttttcttggaattgtgctgttttatcctttaccttgtctacaaaccccttaaaaacgtttttaaaggcttttaagccgtctgtacgttcctaa

SEQ ID NO: 2 - protein, 338 aa, Unknown
  Thermobifida fusca
MQELALKRDLGLSDAEVAELRAAEAEAVELEEELRDSLGSDFGGVYLDADTTEITVAVTDPAAVSRVDADDVTVDVVDFGETALNDFVASLNAIADTADPKVTGWYTDLESDAVVITTLRGGTPAAEELAERAGLDERAVRIVEEDEEPQSLAAIIGGNPYYFGNYRCSIGFSVRQGSQTGFATAGHCGSTGTRVSSPSGTVAGSYFPGRDMGWVRITSADTVTPLVNRYNGGTVTVTGSQEAATGSSVCRSGATTGWRCGTIQSKNQTVRYAEGTVTGLTRTTACAEGGDSGGPWLTGSQAQGVTSGGTGDCRSGGITFFQPINPLLSYFGLQLVTG

SEQ ID NO: 3 - protein, 338 aa, Artificial Sequence
  Thermobifida fusca (F163Y)
MQELALKRDLGLSDAEVAELRAAEAEAVELEEELRDSLGSDFGGVYLDADTTEITVAVTDPAAVSRVDADDVTVDVVDFGETALNDFVASLNAIADTADPKVTGWYTDLESDAVVITTLRGGTPAAEELAERAGLDERAVRIVEEDEEPQSLAAIIGGNPYYYGNYRCSIGFSVRQGSQTGFATAGHCGSTGTRVSSPSGTVAGSYFPGRDMGWVRITSADTVTPLVNRYNGGTVTVTGSQEAATGSSVCRSGATTGWRCGTIQSKNQTVRYAEGTVTGLTRTTACAEGGDSGGPWLTGSQAQGVTSGGTGDCRSGGITFFQPINPLLSYFGLQLVTG

SEQ ID NO: 4 - protein, 338 aa, Artificial Sequence
  Thermobifida fusca (F163Y_N267D)
MQELALKRDLGLSDAEVAELRAAEAEAVELEEELRDSLGSDFGGVYLDADTTEITVAVTDPAAVSRVDADDVTVDVVDFGETALNDFVASLNAIADTADPKVTGWYTDLESDAVVITTLRGGTPAAEELAERAGLDERAVRIVEEDEEPQSLAAIIGGNPYYYGNYRCSIGFSVRQGSQTGFATAGHCGSTGTRVSSPSGTVAGSYFPGRDMGWVRITSADTVTPLVNRYNGGTVTVTGSQEAATGSSVCRSGATTGWRCGTIQSKDQTVRYAEGTVTGLTRTTACAEGGDSGGPWLTGSQAQGVTSGGTGDCRSGGITFFQPINPLLSYFGLQLVTG

SEQ ID NO: 5 - protein, 338 aa, Artificial Sequence
  Thermobifida fusca (F163Y_N267S)
MQELALKRDLGLSDAEVAELRAAEAEAVELEEELRDSLGSDFGGVYLDADTTEITVAVTDPAAVSRVDADDVTVDVVDFGETALNDFVASLNAIADTADPKVTGWYTDLESDAVVITTLRGGTPAAEELAERAGLDERAVRIVEEDEEPQSLAAIIGGNPYYYGNYRCSIGFSVRQGSQTGFATAGHCGSTGTRVSSPSGTVAGSYFPGRDMGWVRITSADTVTPLVNRYNGGTVTVTGSQEAATGSSVCRSGATTGWRCGTIQSKSQTVRYAEGTVTGLTRTTACAEGGDSGGPWLTGSQAQGVTSGGTGDCRSGGITFFQPINPLLSYFGLQLVTG

SEQ ID NO: 6 - protein, 338 aa, Artificial Sequence
  Thermobifida fusca (F163S_N267D)
MQELALKRDLGLSDAEVAELRAAEAEAVELEEELRDSLGSDFGGVYLDADTTEITVAVTDPAAVSRVDADDVTVDVVDFGETALNDFVASLNAIADTADPKVTGWYTDLESDAVVITTLRGGTPAAEELAERAGLDERAVRIVEEDEEPQSLAAIIGGNPYYSGNYRCSIGFSVRQGSQTGFATAGHCGSTGTRVSSPSGTVAGSYFPGRDMGWVRITSADTVTPLVNRYNGGTVTVTGSQEAATGSSVCRSGATTGWRCGTIQSKDQTVRYAEGTVTGLTRTTACAEGGDSGGPWLTGSQAQGVTSGGTGDCRSGGITFFQPINPLLSYFGLQLVTG

SEQ ID NO: 7 - protein, 338 aa, Artificial Sequence
  Thermobifida fusca (F163S_N267T)
MQELALKRDLGLSDAEVAELRAAEAEAVELEEELRDSLGSDFGGVYLDADTTEITVAVTDPAAVSRVDADDVTVDVVDFGETALNDFVASLNAIADTADPKVTGWYTDLESDAVVITTLRGGTPAAEELAERAGLDERAVRIVEEDEEPQSLAAIIGGNPYYSGNYRCSIGFSVRQGSQTGFATAGHCGSTGTRVSSPSGTVAGSYFPGRDMGWVRITSADTVTPLVNRYNGGTVTVTGSQEAATGSSVCRSGATTGWRCGTIQSKTQTVRYAEGTVTGLTRTTACAEGGDSGGPWLTGSQAQGVTSGGTGDCRSGGITFFQPINPLLSYFGLQLVTG

SEQ ID NO: 8 - protein, 338 aa, Artificial Sequence
  Thermobifida fusca (F163A_N267G)
MQELALKRDLGLSDAEVAELRAAEAEAVELEEELRDSLGSDFGGVYLDADTTEITVAVTDPAAVSRVDADDVTVDVVDFGETALNDFVASLNAIADTADPKVTGWYTDLESDAVVITTLRGGTPAAEELAERAGLDERAVRIVEEDEEPQSLAAIIGGNPYYAGNYRCSIGFSVRQGSQTGFATAGHCGSTGTRVSSPSGTVAGSYFPGRDMGWVRITSADTVTPLVNRYNGGTVTVTGSQEAATGSSVCRSGATTGWRCGTIQSKGQTVRYAEGTVTGLTRTTACAEGGDSGGPWLTGSQAQGVTSGGTGDCRSGGITFFQPINPLLSYFGLQLVTG

SEQ ID NO: 9 - protein, 338 aa, Artificial Sequence
  Thermobifida fusca (F163A)
MQELALKRDLGLSDAEVAELRAAEAEAVELEEELRDSLGSDFGGVYLDADTTEITVAVTDPAAVSRVDADDVTVDVVDFGETALNDFVASLNAIADTADPKVTGWYTDLESDAVVITTLRGGTPAAEELAERAGLDERAVRIVEEDEEPQSLAAIIGGNPYYAGNYRCSIGFSVRQGSQTGFATAGHCGSTGTRVSSPSGTVAGSYFPGRDMGWVRITSADTVTPLVNRYNGGTVTVTGSQEAATGSSVCRSGATTGWRCGTIQSKNQTVRYAEGTVTGLTRTTACAEGGDSGGPWLTGSQAQGVTSGGTGDCRSGGITFFQPINPLLSYFGLQLVTG

SEQ ID NO: 10 - protein, 338 aa, Artificial Sequence
  Thermobifida fusca (F163R)
MQELALKRDLGLSDAEVAELRAAEAEAVELEEELRDSLGSDFGGVYLDADTTEITVAVTDPAAVSRVDADDVTVDVVDFGETALNDFVASLNAIADTADPKVTGWYTDLESDAVVITTLRGGTPAAEELAERAGLDERAVRIVEEDEEPQSLAAIIGGNPYYRGNYRCSIGFSVRQGSQTGFATAGHCGSTGTRVSSPSGTVAGSYFPGRDMGWVRITSADTVTPLVNRYNGGTVTVTGSQEAATGSSVCRSGATTGWRCGTIQSKNQTVRYAEGTVTGLTRTTACAEGGDSGGPWLTGSQAQGVTSGGTGDCRSGGITFFQPINPLLSYFGLQLVTG

SEQ ID NO: 11 - DNA, 47 bp, Artificial Sequence
  TAP_mature region_F
aagaagatgaagaaccacagagcttggctgcaattattggtggaaac

SEQ ID NO: 12 - DNA, 44 bp, Artificial Sequence
  TAP_mature region_R
gactgcaggtcgacaagctttcagccggtcactaattgaaggcc

SEQ ID NO: 13 - DNA, 23 bp, Artificial Sequence
  pBE-S-vector-F
aagcttgtcgacctgcagtctag

SEQ ID NO: 14 - DNA, 24 bp, Artificial Sequence
  pBE-S-vector-R
ctgtggttcttcatcttcttccac

SEQ ID NO: 15 - DNA, 37 bp, Artificial Sequence
  TAP_F12Y_F
gtggaaacccgtactattacggaaattacagatgcag

SEQ ID NO: 16 - DNA, 37 bp, Artificial Sequence
  TAP_F12Y_R
ctgcatctgtaatttccgtaatagtacgggtttccac

SEQ ID NO: 17 - DNA, 38 bp, Artificial Sequence
  TAP_N116D_F
ggaactatccaatcaaaagaccaaacggttcgctatgc

SEQ ID NO: 18 - DNA, 38 bp, Artificial Sequence
  TAP_N116D_R
gcatagcgaaccgtttggtcttttgattggatagttcc

SEQ ID NO: 19 - DNA, 37 bp, Artificial Sequence
  Saturation mutagenesis_F_1
gtggaaacccgtactatnnnggaaattacagatgcag

SEQ ID NO: 20 - DNA, 38 bp, Artificial Sequence
  Saturation mutagenesis_R_1
gcatagcgaaccgtttgnnnttttgattggatagttcc

SEQ ID NO: 21 - DNA, 38 bp, Artificial Sequence
  Saturation mutagenesis_F_2
ggaactatccaatcaaaannncaaacggttcgctatgc

SEQ ID NO: 22 - DNA, 37 bp, Artificial Sequence
  Saturation mutagenesis_R_2
ctgcatctgtaatttccnnnatagtacgggtttccac

SEQ ID NO: 23 - DNA, 1017 bp, Artificial Sequence
  Thermobifida fusca (F12Y)
atgcaagagctggcgttgaaacgggacctcggcctctctgacgcagaagtagccgaactccgggctgctgaggcggaagcggtcgagctcgaggaggagctccgcgattcattagggtcagacttcggcggtgtatatctggatgctgacaccaccgaaattacggtcgcggtaaccgacccggcagcggtaagtcgtgtcgacgcggatgatgtcacagttgatgttgtcgatttcggggaaacagctttgaatgattttgtggcttcattaaatgccattgccgacacggcagaccctaaagtcactggatggtataccgatctcgaaagtgatgccgtagtcattacgaccttgcgtggcgggactcctgctgccgaggaacttgctgagagagcgggtctcgacgaaagagccgttcggattgtggaagaagatgaagaaccacagagcttggctgcaattattggtggaaacccgtactattacggaaattacagatgcagtatcgggtttagtgtccgtcagggctctcaaacgggattcgcgaccgcaggccactgcggatccacggggacgcgtgtgtcttctccttcaggaacagttgcaggaagttatttcccgggtcgcgatatgggctgggtgcggattacatcagcagatactgtaacaccactcgtaaatcggtataatgggggaactgttacggtcactgggtcacaagaagctgccaccggatcctccgtttgtcgctctggagcaacaacgggctggcgctgcggaactatccaatcaaaaaaccaaacggttcgctatgcagaagggactgttactggtttaacaagaactacagcctgtgctgaaggtggggattctggagggccatggctcacaggtagccaggcgcaaggggttacaagcggcggaacaggcgattgcagaagtggagggattacctttttccaaccaatcaatccattgcttagctatttcggccttcaattagtgaccggctga

SEQ ID NO: 24 - DNA, 1017 bp, Artificial Sequence
  Thermobifida fusca (F163Y_N267D)
atgcaagagctggcgttgaaacgggacctcggcctctctgacgcagaagtagccgaactccgggctgctgaggcggaagcggtcgagctcgaggaggagctccgcgattcattagggtcagacttcggcggtgtatatctggatgctgacaccaccgaaattacggtcgcggtaaccgacccggcagcggtaagtcgtgtcgacgcggatgatgtcacagttgatgttgtcgatttcggggaaacagctttgaatgattttgtggcttcattaaatgccattgccgacacggcagaccctaaagtcactggatggtataccgatctcgaaagtgatgccgtagtcattacgaccttgcgtggcgggactcctgctgccgaggaacttgctgagagagcgggtctcgacgaaagagccgttcggattgtggaagaagatgaagaaccacagagcttggctgcaattattggtggaaacccgtactattacggaaattacagatgcagtatcgggtttagtgtccgtcagggctctcaaacgggattcgcgaccgcaggccactgcggatccacggggacgcgtgtgtcttctccttcaggaacagttgcaggaagttatttcccgggtcgcgatatgggctgggtgcggattacatcagcagatactgtaacaccactcgtaaatcggtataatgggggaactgttacggtcactgggtcacaagaagctgccaccggatcctccgtttgtcgctctggagcaacaacgggctggcgctgcggaactatccaatcaaaagaccaaacggttcgctatgcagaagggactgttactggtttaacaagaactacagcctgtgctgaaggtggggattctggagggccatggctcacaggtagccaggcgcaaggggttacaagcggcggaacaggcgattgcagaagtggagggattacctttttccaaccaatcaatccattgcttagctatttcggccttcaattagtgaccggctga

SEQ ID NO: 25 - DNA, 1017 bp, Artificial Sequence
  Thermobifida fusca (F163Y_N267S)
atgcaagagctggcgttgaaacgggacctcggcctctctgacgcagaagtagccgaactccgggctgctgaggcggaagcggtcgagctcgaggaggagctccgcgattcattagggtcagacttcggcggtgtatatctggatgctgacaccaccgaaattacggtcgcggtaaccgacccggcagcggtaagtcgtgtcgacgcggatgatgtcacagttgatgttgtcgatttcggggaaacagctttgaatgattttgtggcttcattaaatgccattgccgacacggcagaccctaaagtcactggatggtataccgatctcgaaagtgatgccgtagtcattacgaccttgcgtggcgggactcctgctgccgaggaacttgctgagagagcgggtctcgacgaaagagccgttcggattgtggaagaagatgaagaaccacagagcttggctgcaattattggtggaaacccgtactattacggaaattacagatgcagtatcgggtttagtgtccgtcagggctctcaaacgggattcgcgaccgcaggccactgcggatccacggggacgcgtgtgtcttctccttcaggaacagttgcaggaagttatttcccgggtcgcgatatgggctgggtgcggattacatcagcagatactgtaacaccactcgtaaatcggtataatgggggaactgttacggtcactgggtcacaagaagctgccaccggatcctccgtttgtcgctctggagcaacaacgggctggcgctgcggaactatccaatcaaaaagtcaaacggttcgctatgcagaagggactgttactggtttaacaagaactacagcctgtgctgaaggtggggattctggagggccatggctcacaggtagccaggcgcaaggggttacaagcggcggaacaggcgattgcagaagtggagggattacctttttccaaccaatcaatccattgcttagctatttcggccttcaattagtgaccggctga

SEQ ID NO: 26 - DNA, 1017 bp, Artificial Sequence
  Thermobifida fusca (F163S_N267D)
atgcaagagctggcgttgaaacgggacctcggcctctctgacgcagaagtagccgaactccgggctgctgaggcggaagcggtcgagctcgaggaggagctccgcgattcattagggtcagacttcggcggtgtatatctggatgctgacaccaccgaaattacggtcgcggtaaccgacccggcagcggtaagtcgtgtcgacgcggatgatgtcacagttgatgttgtcgatttcggggaaacagctttgaatgattttgtggcttcattaaatgccattgccgacacggcagaccctaaagtcactggatggtataccgatctcgaaagtgatgccgtagtcattacgaccttgcgtggcgggactcctgctgccgaggaacttgctgagagagcgggtctcgacgaaagagccgttcggattgtggaagaagatgaagaaccacagagcttggctgcaattattggtggaaacccgtactatagtggaaattacagatgcagtatcgggtttagtgtccgtcagggctctcaaacgggattcgcgaccgcaggccactgcggatccacggggacgcgtgtgtcttctccttcaggaacagttgcaggaagttatttcccgggtcgcgatatgggctgggtgcggattacatcagcagatactgtaacaccactcgtaaatcggtataatgggggaactgttacggtcactgggtcacaagaagctgccaccggatcctccgtttgtcgctctggagcaacaacgggctggcgctgcggaactatccaatcaaaagatcaaacggttcgctatgcagaagggactgttactggtttaacaagaactacagcctgtgctgaaggtggggattctggagggccatggctcacaggtagccaggcgcaaggggttacaagcggcggaacaggcgattgcagaagtggagggattacctttttccaaccaatcaatccattgcttagctatttcggccttcaattagtgaccggctga

SEQ ID NO: 27 - DNA, 1017 bp, Artificial Sequence
  Thermobifida fusca (F163S_N267T)
atgcaagagctggcgttgaaacgggacctcggcctctctgacgcagaagtagccgaactccgggctgctgaggcggaagcggtcgagctcgaggaggagctccgcgattcattagggtcagacttcggcggtgtatatctggatgctgacaccaccgaaattacggtcgcggtaaccgacccggcagcggtaagtcgtgtcgacgcggatgatgtcacagttgatgttgtcgatttcggggaaacagctttgaatgattttgtggcttcattaaatgccattgccgacacggcagaccctaaagtcactggatggtataccgatctcgaaagtgatgccgtagtcattacgaccttgcgtggcgggactcctgctgccgaggaacttgctgagagagcgggtctcgacgaaagagccgttcggattgtggaagaagatgaagaaccacagagcttggctgcaattattggtggaaacccgtactatagtggaaattacagatgcagtatcgggtttagtgtccgtcagggctctcaaacgggattcgcgaccgcaggccactgcggatccacggggacgcgtgtgtcttctccttcaggaacagttgcaggaagttatttcccgggtcgcgatatgggctgggtgcggattacatcagcagatactgtaacaccactcgtaaatcggtataatgggggaactgttacggtcactgggtcacaagaagctgccaccggatcctccgtttgtcgctctggagcaacaacgggctggcgctgcggaactatccaatcaaaaactcaaacggttcgctatgcagaagggactgttactggtttaacaagaactacagcctgtgctgaaggtggggattctggagggccatggctcacaggtagccaggcgcaaggggttacaagcggcggaacaggcgattgcagaagtggagggattacctttttccaaccaatcaatccattgcttagctatttcggccttcaattagtgaccggctga

SEQ ID NO: 28 - DNA, 1017 bp, Artificial Sequence
  Thermobifida fusca (F163A_N267G)
atgcaagagctggcgttgaaacgggacctcggcctctctgacgcagaagtagccgaactccgggctgctgaggcggaagcggtcgagctcgaggaggagctccgcgattcattagggtcagacttcggcggtgtatatctggatgctgacaccaccgaaattacggtcgcggtaaccgacccggcagcggtaagtcgtgtcgacgcggatgatgtcacagttgatgttgtcgatttcggggaaacagctttgaatgattttgtggcttcattaaatgccattgccgacacggcagaccctaaagtcactggatggtataccgatctcgaaagtgatgccgtagtcattacgaccttgcgtggcgggactcctgctgccgaggaacttgctgagagagcgggtctcgacgaaagagccgttcggattgtggaagaagatgaagaaccacagagcttggctgcaattattggtggaaacccgtactatgctggaaattacagatgcagtatcgggtttagtgtccgtcagggctctcaaacgggattcgcgaccgcaggccactgcggatccacggggacgcgtgtgtcttctccttcaggaacagttgcaggaagttatttcccgggtcgcgatatgggctgggtgcggattacatcagcagatactgtaacaccactcgtaaatcggtataatgggggaactgttacggtcactgggtcacaagaagctgccaccggatcctccgtttgtcgctctggagcaacaacgggctggcgctgcggaactatccaatcaaaaggtcaaacggttcgctatgcagaagggactgttactggtttaacaagaactacagcctgtgctgaaggtggggattctggagggccatggctcacaggtagccaggcgcaaggggttacaagcggcggaacaggcgattgcagaagtggagggattacctttttccaaccaatcaatccattgcttagctatttcggccttcaattagtgaccggctga

SEQ ID NO: 29 - DNA, 1017 bp, Artificial Sequence
  Thermobifida fusca (F163A)
atgcaagagctggcgttgaaacgggacctcggcctctctgacgcagaagtagccgaactccgggctgctgaggcggaagcggtcgagctcgaggaggagctccgcgattcattagggtcagacttcggcggtgtatatctggatgctgacaccaccgaaattacggtcgcggtaaccgacccggcagcggtaagtcgtgtcgacgcggatgatgtcacagttgatgttgtcgatttcggggaaacagctttgaatgattttgtggcttcattaaatgccattgccgacacggcagaccctaaagtcactggatggtataccgatctcgaaagtgatgccgtagtcattacgaccttgcgtggcgggactcctgctgccgaggaacttgctgagagagcgggtctcgacgaaagagccgttcggattgtggaagaagatgaagaaccacagagcttggctgcaattattggtggaaacccgtactatgctggaaattacagatgcagtatcgggtttagtgtccgtcagggctctcaaacgggattcgcgaccgcaggccactgcggatccacggggacgcgtgtgtcttctccttcaggaacagttgcaggaagttatttcccgggtcgcgatatgggctgggtgcggattacatcagcagatactgtaacaccactcgtaaatcggtataatgggggaactgttacggtcactgggtcacaagaagctgccaccggatcctccgtttgtcgctctggagcaacaacgggctggcgctgcggaactatccaatcaaaaaatcaaacggttcgctatgcagaagggactgttactggtttaacaagaactacagcctgtgctgaaggtggggattctggagggccatggctcacaggtagccaggcgcaaggggttacaagcggcggaacaggcgattgcagaagtggagggattacctttttccaaccaatcaatccattgcttagctatttcggccttcaattagtgaccggctga

SEQ ID NO: 30 - DNA, 1017 bp, Artificial Sequence
  Thermobifida fusca (F163R)
atgcaagagctggcgttgaaacgggacctcggcctctctgacgcagaagtagccgaactccgggctgctgaggcggaagcggtcgagctcgaggaggagctccgcgattcattagggtcagacttcggcggtgtatatctggatgctgacaccaccgaaattacggtcgcggtaaccgacccggcagcggtaagtcgtgtcgacgcggatgatgtcacagttgatgttgtcgatttcggggaaacagctttgaatgattttgtggcttcattaaatgccattgccgacacggcagaccctaaagtcactggatggtataccgatctcgaaagtgatgccgtagtcattacgaccttgcgtggcgggactcctgctgccgaggaacttgctgagagagcgggtctcgacgaaagagccgttcggattgtggaagaagatgaagaaccacagagcttggctgcaattattggtggaaacccgtactatagaggaaattacagatgcagtatcgggtttagtgtccgtcagggctctcaaacgggattcgcgaccgcaggccactgcggatccacggggacgcgtgtgtcttctccttcaggaacagttgcaggaagttatttcccgggtcgcgatatgggctgggtgcggattacatcagcagatactgtaacaccactcgtaaatcggtataatgggggaactgttacggtcactgggtcacaagaagctgccaccggatcctccgtttgtcgctctggagcaacaacgggctggcgctgcggaactatccaatcaaaaaatcaaacggttcgctatgcagaagggactgttactggtttaacaagaactacagcctgtgctgaaggtggggattctggagggccatggctcacaggtagccaggcgcaaggggttacaagcggcggaacaggcgattgcagaagtggagggattacctttttccaaccaatcaatccattgcttagctatttcggccttcaattagtgaccggctga

SEQ ID NO: 31 - protein, 187 aa, Unknown
  Thermobifida fusca_mature region
LAAIIGGNPYYFGNYRCSIGFSVRQGSQTGFATAGHCGSTGTRVSSPSGTVAGSYFPGRDMGWVRITSADTVTPLVNRYNGGTVTVTGSQEAATGSSVCRSGATTGWRCGTIQSKNQTVRYAEGTVTGLTRTTACAEGGDSGGPWLTGSQAQGVTSGGTGDCRSGGITFFQPINPLLSYFGLQLVTG

SEQ ID NO: 32 - protein, 187 aa, Artificial Sequence
  Thermobifida fusca_mature region (F12Y)
LAAIIGGNPYYYGNYRCSIGFSVRQGSQTGFATAGHCGSTGTRVSSPSGTVAGSYFPGRDMGWVRITSADTVTPLVNRYNGGTVTVTGSQEAATGSSVCRSGATTGWRCGTIQSKNQTVRYAEGTVTGLTRTTACAEGGDSGGPWLTGSQAQGVTSGGTGDCRSGGITFFQPINPLLSYFGLQLVTG

SEQ ID NO: 33 - protein, 187 aa, Artificial Sequence
  Thermobifida fusca_mature region (F12Y_N116D)
LAAIIGGNPYYYGNYRCSIGFSVRQGSQTGFATAGHCGSTGTRVSSPSGTVAGSYFPGRDMGWVRITSADTVTPLVNRYNGGTVTVTGSQEAATGSSVCRSGATTGWRCGTIQSKDQTVRYAEGTVTGLTRTTACAEGGDSGGPWLTGSQAQGVTSGGTGDCRSGGITFFQPINPLLSYFGLQLVTG

SEQ ID NO: 34 - protein, 187 aa, Artificial Sequence
  Thermobifida fusca_mature region (F12Y_N116S)
LAAIIGGNPYYYGNYRCSIGFSVRQGSQTGFATAGHCGSTGTRVSSPSGTVAGSYFPGRDMGWVRITSADTVTPLVNRYNGGTVTVTGSQEAATGSSVCRSGATTGWRCGTIQSKSQTVRYAEGTVTGLTRTTACAEGGDSGGPWLTGSQAQGVTSGGTGDCRSGGITFFQPINPLLSYFGLQLVTG

SEQ ID NO: 35 - protein, 187 aa, Artificial Sequence
  Thermobifida fusca_mature region (F12S_N116D)
LAAIIGGNPYYSGNYRCSIGFSVRQGSQTGFATAGHCGSTGTRVSSPSGTVAGSYFPGRDMGWVRITSADTVTPLVNRYNGGTVTVTGSQEAATGSSVCRSGATTGWRCGTIQSKDQTVRYAEGTVTGLTRTTACAEGGDSGGPWLTGSQAQGVTSGGTGDCRSGGITFFQPINPLLSYFGLQLVTG

SEQ ID NO: 36 - protein, 187 aa, Artificial Sequence
  Thermobifida fusca_mature region (F12S_N116T)
LAAIIGGNPYYSGNYRCSIGFSVRQGSQTGFATAGHCGSTGTRVSSPSGTVAGSYFPGRDMGWVRITSADTVTPLVNRYNGGTVTVTGSQEAATGSSVCRSGATTGWRCGTIQSKTQTVRYAEGTVTGLTRTTACAEGGDSGGPWLTGSQAQGVTSGGTGDCRSGGITFFQPINPLLSYFGLQLVTG

SEQ ID NO: 37 - protein, 187 aa, Artificial Sequence
  Thermobifida fusca_mature region (F12A_N116G)
LAAIIGGNPYYAGNYRCSIGFSVRQGSQTGFATAGHCGSTGTRVSSPSGTVAGSYFPGRDMGWVRITSADTVTPLVNRYNGGTVTVTGSQEAATGSSVCRSGATTGWRCGTIQSKGQTVRYAEGTVTGLTRTTACAEGGDSGGPWLTGSQAQGVTSGGTGDCRSGGITFFQPINPLLSYFGLQLVTG

SEQ ID NO: 38 - protein, 187 aa, Artificial Sequence
  Thermobifida fusca_mature region (F12A)
LAAIIGGNPYYAGNYRCSIGFSVRQGSQTGFATAGHCGSTGTRVSSPSGTVAGSYFPGRDMGWVRITSADTVTPLVNRYNGGTVTVTGSQEAATGSSVCRSGATTGWRCGTIQSKNQTVRYAEGTVTGLTRTTACAEGGDSGGPWLTGSQAQGVTSGGTGDCRSGGITFFQPINPLLSYFGLQLVTG

SEQ ID NO: 39 - protein, 187 aa, Artificial Sequence
  Thermobifida fusca_mature region (F12R)
LAAIIGGNPYYRGNYRCSIGFSVRQGSQTGFATAGHCGSTGTRVSSPSGTVAGSYFPGRDMGWVRITSADTVTPLVNRYNGGTVTVTGSQEAATGSSVCRSGATTGWRCGTIQSKNQTVRYAEGTVTGLTRTTACAEGGDSGGPWLTGSQAQGVTSGGTGDCRSGGITFFQPINPLLSYFGLQLVTG

SEQ ID NO: 40 - protein, 368 aa, Unknown
  Thermobifida fusca
MNHSSRRTTSLLFTAALAATALVAATTPASAQELALKRDLGLSDAEVAELRAAEAEAVELEEELRDSLGSDFGGVYLDADTTEITVAVTDPAAVSRVDADDVTVDVVDFGETALNDFVASLNAIADTADPKVTGWYTDLESDAVVITTLRGGTPAAEELAERAGLDERAVRIVEEDEEPQSLAAIIGGNPYYFGNYRCSIGFSVRQGSQTGFATAGHCGSTGTRVSSPSGTVAGSYFPGRDMGWVRITSADTVTPLVNRYNGGTVTVTGSQEAATGSSVCRSGATTGWRCGTIQSKNQTVRYAEGTVTGLTRTTACAEGGDSGGPWLTGSQAQGVTSGGTGDCRSGGITFFQPINPLLSYFGLQLVTG

SEQ ID NO: 41 - DNA, 564 bp, Artificial Sequence
  Thermobifida fusca_mature region (F12Y)
ttggctgcaattattggtggaaacccgtactattacggaaattacagatgcagtatcgggtttagtgtccgtcagggctctcaaacgggattcgcgaccgcaggccactgcggatccacggggacgcgtgtgtcttctccttcaggaacagttgcaggaagttatttcccgggtcgcgatatgggctgggtgcggattacatcagcagatactgtaacaccactcgtaaatcggtataatgggggaactgttacggtcactgggtcacaagaagctgccaccggatcctccgtttgtcgctctggagcaacaacgggctggcgctgcggaactatccaatcaaaaaaccaaacggttcgctatgcagaagggactgttactggtttaacaagaactacagcctgtgctgaaggtggggattctggagggccatggctcacaggtagccaggcgcaaggggttacaagcggcggaacaggcgattgcagaagtggagggattacctttttccaaccaatcaatccattgcttagctatttcggccttcaattagtgaccggctga

SEQ ID NO: 42 - DNA, 564 bp, Artificial Sequence
  Thermobifida fusca_mature region (F12Y_N116D)
ttggctgcaattattggtggaaacccgtactattacggaaattacagatgcagtatcgggtttagtgtccgtcagggctctcaaacgggattcgcgaccgcaggccactgcggatccacggggacgcgtgtgtcttctccttcaggaacagttgcaggaagttatttcccgggtcgcgatatgggctgggtgcggattacatcagcagatactgtaacaccactcgtaaatcggtataatgggggaactgttacggtcactgggtcacaagaagctgccaccggatcctccgtttgtcgctctggagcaacaacgggctggcgctgcggaactatccaatcaaaagaccaaacggttcgctatgcagaagggactgttactggtttaacaagaactacagcctgtgctgaaggtggggattctggagggccatggctcacaggtagccaggcgcaaggggttacaagcggcggaacaggcgattgcagaagtggagggattacctttttccaaccaatcaatccattgcttagctatttcggccttcaattagtgaccggctga

SEQ ID NO: 43 - DNA, 564 bp, Artificial Sequence
  Thermobifida fusca_mature region (F12Y_N116S)
ttggctgcaattattggtggaaacccgtactattacggaaattacagatgcagtatcgggtttagtgtccgtcagggctctcaaacgggattcgcgaccgcaggccactgcggatccacggggacgcgtgtgtcttctccttcaggaacagttgcaggaagttatttcccgggtcgcgatatgggctgggtgcggattacatcagcagatactgtaacaccactcgtaaatcggtataatgggggaactgttacggtcactgggtcacaagaagctgccaccggatcctccgtttgtcgctctggagcaacaacgggctggcgctgcggaactatccaatcaaaaagtcaaacggttcgctatgcagaagggactgttactggtttaacaagaactacagcctgtgctgaaggtggggattctggagggccatggctcacaggtagccaggcgcaaggggttacaagcggcggaacaggcgattgcagaagtggagggattacctttttccaaccaatcaatccattgcttagctatttcggccttcaattagtgaccggctga

SEQ ID NO: 44 - DNA, 564 bp, Artificial Sequence
  Thermobifida fusca_mature region (F12S_N116D)
ttggctgcaattattggtggaaacccgtactatagtggaaattacagatgcagtatcgggtttagtgtccgtcagggctctcaaacgggattcgcgaccgcaggccactgcggatccacggggacgcgtgtgtcttctccttcaggaacagttgcaggaagttatttcccgggtcgcgatatgggctgggtgcggattacatcagcagatactgtaacaccactcgtaaatcggtataatgggggaactgttacggtcactgggtcacaagaagctgccaccggatcctccgtttgtcgctctggagcaacaacgggctggcgctgcggaactatccaatcaaaagatcaaacggttcgctatgcagaagggactgttactggtttaacaagaactacagcctgtgctgaaggtggggattctggagggccatggctcacaggtagccaggcgcaaggggttacaagcggcggaacaggcgattgcagaagtggagggattacctttttccaaccaatcaatccattgcttagctatttcggccttcaattagtgaccggctga

SEQ ID NO: 45 - DNA, 564 bp, Artificial Sequence
  Thermobifida fusca_mature region (F12S_N116T)
ttggctgcaattattggtggaaacccgtactatagtggaaattacagatgcagtatcgggtttagtgtccgtcagggctctcaaacgggattcgcgaccgcaggccactgcggatccacggggacgcgtgtgtcttctccttcaggaacagttgcaggaagttatttcccgggtcgcgatatgggctgggtgcggattacatcagcagatactgtaacaccactcgtaaatcggtataatgggggaactgttacggtcactgggtcacaagaagctgccaccggatcctccgtttgtcgctctggagcaacaacgggctggcgctgcggaactatccaatcaaaaactcaaacggttcgctatgcagaagggactgttactggtttaacaagaactacagcctgtgctgaaggtggggattctggagggccatggctcacaggtagccaggcgcaaggggttacaagcggcggaacaggcgattgcagaagtggagggattacctttttccaaccaatcaatccattgcttagctatttcggccttcaattagtgaccggctga

SEQ ID NO: 46 - DNA, 564 bp, Artificial Sequence
  Thermobifida fusca_mature region (F12A_N116G)
ttggctgcaattattggtggaaacccgtactatgctggaaattacagatgcagtatcgggtttagtgtccgtcagggctctcaaacgggattcgcgaccgcaggccactgcggatccacggggacgcgtgtgtcttctccttcaggaacagttgcaggaagttatttcccgggtcgcgatatgggctgggtgcggattacatcagcagatactgtaacaccactcgtaaatcggtataatgggggaactgttacggtcactgggtcacaagaagctgccaccggatcctccgtttgtcgctctggagcaacaacgggctggcgctgcggaactatccaatcaaaaggtcaaacggttcgctatgcagaagggactgttactggtttaacaagaactacagcctgtgctgaaggtggggattctggagggccatggctcacaggtagccaggcgcaaggggttacaagcggcggaacaggcgattgcagaagtggagggattacctttttccaaccaatcaatccattgcttagctatttcggccttcaattagtgaccggctga

SEQ ID NO: 47 - DNA, 564 bp, Artificial Sequence
  Thermobifida fusca_mature region (F12A)
ttggctgcaattattggtggaaacccgtactatgctggaaattacagatgcagtatcgggtttagtgtccgtcagggctctcaaacgggattcgcgaccgcaggccactgcggatccacggggacgcgtgtgtcttctccttcaggaacagttgcaggaagttatttcccgggtcgcgatatgggctgggtgcggattacatcagcagatactgtaacaccactcgtaaatcggtataatgggggaactgttacggtcactgggtcacaagaagctgccaccggatcctccgtttgtcgctctggagcaacaacgggctggcgctgcggaactatccaatcaaaaaatcaaacggttcgctatgcagaagggactgttactggtttaacaagaactacagcctgtgctgaaggtggggattctggagggccatggctcacaggtagccaggcgcaaggggttacaagcggcggaacaggcgattgcagaagtggagggattacctttttccaaccaatcaatccattgcttagctatttcggccttcaattagtgaccggctga

SEQ ID NO: 48 - DNA, 564 bp, Artificial Sequence
  Thermobifida fusca_mature region (F12R)
ttggctgcaattattggtggaaacccgtactatagaggaaattacagatgcagtatcgggtttagtgtccgtcagggctctcaaacgggattcgcgaccgcaggccactgcggatccacggggacgcgtgtgtcttctccttcaggaacagttgcaggaagttatttcccgggtcgcgatatgggctgggtgcggattacatcagcagatactgtaacaccactcgtaaatcggtataatgggggaactgttacggtcactgggtcacaagaagctgccaccggatcctccgtttgtcgctctggagcaacaacgggctggcgctgcggaactatccaatcaaaaaatcaaacggttcgctatgcagaagggactgttactggtttaacaagaactacagcctgtgctgaaggtggggattctggagggccatggctcacaggtagccaggcgcaaggggttacaagcggcggaacaggcgattgcagaagtggagggattacctttttccaaccaatcaatccattgcttagctatttcggccttcaattagtgaccggctga

SEQ ID NO: 49 - protein, 187 aa, Unknown
  Thermobifida cellulosilytica
FADVIGGNPYYFGGYRCSIGFSVRKGSDTGFATAGHCGETGTLTRSPEGVVAGSYFPGRDMGWVRLTGADTVTPLVNRYDGGTVTVTGSQEAVTGSSVCRSGSTTGWRCGIIQSKNQTVRYAEGTVTGLTRTTACAEAGDSGGPWLTGSQAQGVTSGGSGNCRTGGITYFQPINPLLSYFGLELVTG

SEQ ID NO: 50 - protein, 187 aa, Unknown
  Thermobifida halotolerans
FTDIIGGNPYYFDGYRCSIGFSVRRGSESGFATAGHCGEEGTETSDPEGTVAGAYFPGRDMGWVRITDADTVTPLVNRYNGENVTVAGSREAATGSSVCRSGSTTGWRCGTIRSKNQTVRYIEGTVTGLTRTTACAEGGDSGGPWLTGSQGQGVTSGGSGNCTLGGVTYFQPLNPLLSHFDLDLVTG

SEQ ID NO: 51 - protein, 187 aa, Unknown
  Actinorugispora endophytica
LANVIGGNAYYFGGYRCSVGFSVRHSSGPGFATAGHCGDVGTRTTSPTGTIAGSYFPGRDMGWVRITSADTVTPLVNRYNGSYITVTGSSEAANGSSVCRSGSTTGWHCGTIQSKNQTVNYAEGSVAGLTRTTACAEGGDSGGSWLTGTQAQGVTSGGSGNCTWGGTTYFQPINPLLSYFNLTLVTG

SEQ ID NO: 52 - protein, 183 aa, Unknown
  Spinactinospora alkalitolerans
FADIIGGNAYYPGSSRCSIGFAVQGGFVTAGHCGSTGTRTSSPSGTVAGSWFPGRDMGWVRTGSGDTPRPWVNNYRGGYVTVAGSQEAGIGSSVCRSGSTTGWHCGTIQSKNQTVRYSQGSVYGLTRTSACAEPGDSGGSWVTGNQAQGVTSGGSGNCTWGGTTYFQPVNPILSQYGLRLVTG

SEQ ID NO: 53 - protein, 186 aa, Unknown
  Nocardiopsis composta
FGDIVGGNAYYPGGSRCSIGFSVQGGFATAGHCGSQGTRVTGGAGESGTVAGSIFPGRDMGWVRVNSGWNPSPYVNNYSGGRVLVTGSQEASVGASVCRSGSTTGWRCGTIQAKNQTVRYPEGTVNGLTRTTACAEPGDSGGSWLSGNQAQGVTSGGSGNCSSGGTTFFQPLNPILSQWGLTLTTG

SEQ ID NO: 54 - protein, 186 aa, Unknown
  Nocardiopsis potens
FGDIVGGNAYYPGGSRCSIGFSVQGGFATAGHCGSQGTRVTGGAGESGTVAGSIFPGRDMGWVRVNSGWNPSPYVNNYSGGRVLVTGSQEASVGASICRSGSTTGWHCGTIQAKNQTVRYPQGTVNGLTRTNVCAEPGDSGGSWISGSQAQGVTSGGSGNCSTGGTTFYQPINPILSQWGLTLTTG

SEQ ID NO: 55 - protein, 187 aa, Artificial Sequence
  Thermobifida cellulosilytica_F12Y
FADVIGGNPYYYGGYRCSIGFSVRKGSDTGFATAGHCGETGTLTRSPEGVVAGSYFPGRDMGWVRLTGADTVTPLVNRYDGGTVTVTGSQEAVTGSSVCRSGSTTGWRCGIIQSKNQTVRYAEGTVTGLTRTTACAEAGDSGGPWLTGSQAQGVTSGGSGNCRTGGITYFQPINPLLSYFGLELVTG

SEQ ID NO: 56 - protein, 187 aa, Artificial Sequence
  Thermobifida cellulosilytica_F12YN116D
FADVIGGNPYYYGGYRCSIGFSVRKGSDTGFATAGHCGETGTLTRSPEGVVAGSYFPGRDMGWVRLTGADTVTPLVNRYDGGTVTVTGSQEAVTGSSVCRSGSTTGWRCGIIQSKDQTVRYAEGTVTGLTRTTACAEAGDSGGPWLTGSQAQGVTSGGSGNCRTGGITYFQPINPLLSYFGLELVTG

SEQ ID NO: 57 - protein, 187 aa, Artificial Sequence
  Thermobifida halotolerans_F12Y
FTDIIGGNPYYYDGYRCSIGFSVRRGSESGFATAGHCGEEGTETSDPEGTVAGAYFPGRDMGWVRITDADTVTPLVNRYNGENVTVAGSREAATGSSVCRSGSTTGWRCGTIRSKNQTVRYIEGTVTGLTRTTACAEGGDSGGPWLTGSQGQGVTSGGSGNCTLGGVTYFQPLNPLLSHFDLDLVTG

SEQ ID NO: 58 - protein, 187 aa, Artificial Sequence
  Thermobifida halotolerans_F12YN116D
FTDIIGGNPYYYDGYRCSIGFSVRRGSESGFATAGHCGEEGTETSDPEGTVAGAYFPGRDMGWVRITDADTVTPLVNRYNGENVTVAGSREAATGSSVCRSGSTTGWRCGTIRSKDQTVRYIEGTVTGLTRTTACAEGGDSGGPWLTGSQGQGVTSGGSGNCTLGGVTYFQPLNPLLSHFDLDLVTG

SEQ ID NO: 59 - protein, 187 aa, Artificial Sequence
  Actinorugispora endophytica_F12Y
LANVIGGNAYYYGGYRCSVGFSVRHSSGPGFATAGHCGDVGTRTTSPTGTIAGSYFPGRDMGWVRITSADTVTPLVNRYNGSYITVTGSSEAANGSSVCRSGSTTGWHCGTIQSKNQTVNYAEGSVAGLTRTTACAEGGDSGGSWLTGTQAQGVTSGGSGNCTWGGTTYFQPINPLLSYFNLTLVTG

SEQ ID NO: 60 - protein, 187 aa, Artificial Sequence
  Actinorugispora endophytica_F12YN116D
LANVIGGNAYYYGGYRCSVGFSVRHSSGPGFATAGHCGDVGTRTTSPTGTIAGSYFPGRDMGWVRITSADTVTPLVNRYNGSYITVTGSSEAANGSSVCRSGSTTGWHCGTIQSKDQTVNYAEGSVAGLTRTTACAEGGDSGGSWLTGTQAQGVTSGGSGNCTWGGTTYFQPINPLLSYFNLTLVTG

SEQ ID NO: 61 - protein, 183 aa, Artificial Sequence
  Spinactinospora alkalitolerans_F12Y
FADIIGGNAYYYGSSRCSIGFAVQGGFVTAGHCGSTGTRTSSPSGTVAGSWFPGRDMGWVRTGSGDTPRPWVNNYRGGYVTVAGSQEAGIGSSVCRSGSTTGWHCGTIQSKNQTVRYSQGSVYGLTRTSACAEPGDSGGSWVTGNQAQGVTSGGSGNCTWGGTTYFQPVNPILSQYGLRLVTG

SEQ ID NO: 62 - protein, 183 aa, Artificial Sequence
  Spinactinospora alkalitolerans_F12YN116D
FADIIGGNAYYYGSSRCSIGFAVQGGFVTAGHCGSTGTRTSSPSGTVAGSWFPGRDMGWVRTGSGDTPRPWVNNYRGGYVTVAGSQEAGIGSSVCRSGSTTGWHCGTIQSKDQTVRYSQGSVYGLTRTSACAEPGDSGGSWVTGNQAQGVTSGGSGNCTWGGTTYFQPVNPILSQYGLRLVTG

SEQ ID NO: 63 - protein, 186 aa, Artificial Sequence
  Nocardiopsis composta_F12Y
FGDIVGGNAYYYGGSRCSIGFSVQGGFATAGHCGSQGTRVTGGAGESGTVAGSIFPGRDMGWVRVNSGWNPSPYVNNYSGGRVLVTGSQEASVGASVCRSGSTTGWRCGTIQAKNQTVRYPEGTVNGLTRTTACAEPGDSGGSWLSGNQAQGVTSGGSGNCSSGGTTFFQPLNPILSQWGLTLTTG

SEQ ID NO: 64 - protein, 186 aa, Artificial Sequence
  Nocardiopsis composta_F12YN116D
FGDIVGGNAYYYGGSRCSIGFSVQGGFATAGHCGSQGTRVTGGAGESGTVAGSIFPGRDMGWVRVNSGWNPSPYVNNYSGGRVLVTGSQEASVGASVCRSGSTTGWRCGTIQAKDQTVRYPEGTVNGLTRTTACAEPGDSGGSWLSGNQAQGVTSGGSGNCSSGGTTFFQPLNPILSQWGLTLTTG

SEQ ID NO: 65 - protein, 186 aa, Artificial Sequence
  Nocardiopsis potens_F12Y
FGDIVGGNAYYYGGSRCSIGFSVQGGFATAGHCGSQGTRVTGGAGESGTVAGSIFPGRDMGWVRVNSGWNPSPYVNNYSGGRVLVTGSQEASVGASICRSGSTTGWHCGTIQAKNQTVRYPQGTVNGLTRTNVCAEPGDSGGSWISGSQAQGVTSGGSGNCSTGGTTFYQPINPILSQWGLTLTTG

SEQ ID NO: 66 - protein, 186 aa, Artificial Sequence
  Nocardiopsis potens_F12YN116D
FGDIVGGNAYYYGGSRCSIGFSVQGGFATAGHCGSQGTRVTGGAGESGTVAGSIFPGRDMGWVRVNSGWNPSPYVNNYSGGRVLVTGSQEASVGASICRSGSTTGWHCGTIQAKDQTVRYPQGTVNGLTRTNVCAEPGDSGGSWISGSQAQGVTSGGSGNCSTGGTTFYQPINPILSQWGLTLTTG

SEQ ID NO: 67 - protein, 374 aa, Unknown
  Thermobifida cellulosilytica
MNRPSTRRTVRALLTAALAATALTAPAAPSLAQEASQEAALTRDLDLTGTEVALLRAAESEAMDREEELSAVLGSDFGGVYLAPETGEVTVAVTDPAAVPVVEQSGATAQVVTFGETALNDFVDSLNAVADRADEQITGWYTDLAADTVVITAFPGGSAAAEELAALAGVDERAVRVTESAARPQLFADVIGGNPYYFGGYRCSIGFSVRKGSDTGFATAGHCGETGTLTRSPEGVVAGSYFPGRDMGWVRLTGADTVTPLVNRYDGGTVTVTGSQEAVTGSSVCRSGSTTGWRCGIIQSKNQTVRYAEGTVTGLTRTTACAEAGDSGGPWLTGSQAQGVTSGGSGNCRTGGITYFQPINPLLSYFGLELVTGA

SEQ ID NO: 68 - protein, 354 aa, Unknown
  Thermobifida halotolerans
MVATALTASATPASADRHDALKRDLGLTDSEVARLRTAETEAMDREAELRDTLGSDFGGVHLDAASGELTIAVTDPEAVPTVERAGANAEVVTFGESALNGFVDSLNSVADQADEQVTGWYADIADDSVVITVREGGTAAAEALVARAGVDERAVRVTKSDERPQLFTDIIGGNPYYFDGYRCSIGFSVRRGSESGFATAGHCGEEGTETSDPEGTVAGAYFPGRDMGWVRITDADTVTPLVNRYNGENVTVAGSREAATGSSVCRSGSTTGWRCGTIRSKNQTVRYIEGTVTGLTRTTACAEGGDSGGPWLTGSQGQGVTSGGSGNCTLGGVTYFQPLNPLLSHFDLDLVTGA

SEQ ID NO: 69 - protein, 383 aa, Unknown
  Actinorugispora endophytica
MKRSSVFRALGGTILTAGLVITAAPFASAAPVHTETTPTAAEAGDQLSALKRDLGLSTAEVEELQAAEAEAMDVEEGLRETLGSDFGGAHFDIDSGELTVSVTDAAAVSTVEAAGANAEVVDFGEPALDAIVEDLNTVAEEADDSVTGWYVDTADDSVVITVLEGDTEAAEALVAEADVDGKAVRVEETTEQPKLLANVIGGNAYYFGGYRCSVGFSVRHSSGPGFATAGHCGDVGTRTTSPTGTIAGSYFPGRDMGWVRITSADTVTPLVNRYNGSYITVTGSSEAANGSSVCRSGSTTGWHCGTIQSKNQTVNYAEGSVAGLTRTTACAEGGDSGGSWLTGTQAQGVTSGGSGNCTWGGTTYFQPINPLLSYFNLTLVTGA

SEQ ID NO: 70 - protein, 375 aa, Unknown
  Spinactinospora alkalitolerans
MRKSPIIRAVGGAAITFGLVIAAAPFASADSGSETTAGSVGQLGAMQRDLGLSATEATALLDQEEQARTLEGELRETLGGDFGGAVFDIESGELTVSVTDEDAVDEVREAGAEAEVVTYGEQRLDAIVDDLNATEDTADESVTGWYVDTADDSVVVTVMEGEEAAAEKLIATADVEGTAVRVEETTEQPETFADIIGGNAYYPGSSRCSIGFAVQGGFVTAGHCGSTGTRTSSPSGTVAGSWFPGRDMGWVRTGSGDTPRPWVNNYRGGYVTVAGSQEAGIGSSVCRSGSTTGWHCGTIQSKNQTVRYSQGSVYGLTRTSACAEPGDSGGSWVTGNQAQGVTSGGSGNCTWGGTTYFQPVNPILSQYGLRLVTGA

SEQ ID NO: 71 - protein, 376 aa, Unknown
  Nocardiopsis composta
MRKSPYIPLLGASVLALGMIAASPTAASADEATDSSPARALASGLDMSTAQAAELLDAEAQARTAEQEARELAGASFAGAVFDADTRKLTVSVTDAAAAEAVQATGAETRVVEASADELDAAVADLNAEERGLGSEIDGVTGWYVDQAANELVVTVLDGETEAAETLLDEAGVDSVPVRVDQGAEQPETFGDIVGGNAYYPGGSRCSIGFSVQGGFATAGHCGSQGTRVTGGAGESGTVAGSIFPGRDMGWVRVNSGWNPSPYVNNYSGGRVLVTGSQEASVGASVCRSGSTTGWRCGTIQAKNQTVRYPEGTVNGLTRTTACAEPGDSGGSWLSGNQAQGVTSGGSGNCSSGGTTFFQPLNPILSQWGLTLTTGA

SEQ ID NO: 72 - protein, 376 aa, Unknown
  Nocardiopsis potens
MRKSPYISFLGASALALGMIAASPAAASADEAADTSPAEALASGLDMSASQAADLLDAEAEARGTEAEAREAAGGSFAGAVFDAESQVLTVSVTDAAAAEAVEATGAETRVVEASEDELDSAVSDLNAEESSLGSAIEGVTGWYVDPAANEVVVTVLDGETAAAETLLDEAGVDGVPVRIDEGAEQPETFGDIVGGNAYYPGGSRCSIGFSVQGGFATAGHCGSQGTRVTGGAGESGTVAGSIFPGRDMGWVRVNSGWNPSPYVNNYSGGRVLVTGSQEASVGASICRSGSTTGWHCGTIQAKNQTVRYPQGTVNGLTRTNVCAEPGDSGGSWISGSQAQGVTSGGSGNCSTGGTTFYQPINPILSQWGLTLTTGA